European Patent Specification EP 3 735 979 B1, published August 13, 2025. Title: Methods for wound healing. Applicant: Phillipson, Mia Roos, Stefan Vagesjo, Evelina. The sequence listing filed with the application follows.

SEQUENCE LISTING (26 sequences)

SEQ ID NO: 1 - DNA, 299 bp, Mus musculus
  CDS (3)..(293)
ccatggcaaaattttggaagaaagcactattaacaattgcagccttaacagtcggcacctccgcaggaattacaagcgtttctgccaaaccggtaagtttgtcatatcgatgtccatgccggtttttcgaatctcatattgcacgcgctaatgtcaaacacttaaagattcttaatactcctaattgtgctttgcagattgttgcacgtttaaagaataacaatcgtcaagtttgtatcgatccaaagcttaaatggattcaagagtacttagaaaaggccttaaacaaataactcgag

SEQ ID NO: 2 - protein, 96 aa, Mus musculus
MAKFWKKALLTIAALTVGTSAGITSVSAKPVSLSYRCPCRFFESHIARANVKHLKILNTPNCALQIVARLKNNNRQVCIDPKLKWIQEYLEKALNK

SEQ ID NO: 3 - protein, 89 aa, Mus musculus
MDAKVVAVLALVLAALCISDGKPVSLSYRCPCRFFESHIARANVKHLKILNTPNCALQIVARLKNNNRQVCIDPKLKWIQEYLEKALNK

SEQ ID NO: 4 - DNA, 299 bp, Homo sapiens
  CDS (3)..(293)
ccatggcaaaattttggaagaaagcactattaacaattgcagccttaacagtcggcacctccgcaggaattacaagcgtttctgccaaaccggtaagtttgtcatatcgatgtccatgccggtttttcgaatctcatgttgcacgcgctaatgtcaaacacttaaagattcttaatactcctaattgtgctttgcagattgttgcacgtttaaagaataacaatcgtcaagtttgtatcgatccaaagcttaaatggattcaagagtacttagaaaaggccttaaacaaataactcgag

SEQ ID NO: 5 - protein, 96 aa, Homo sapiens
MAKFWKKALLTIAALTVGTSAGITSVSAKPVSLSYRCPCRFFESHVARANVKHLKILNTPNCALQIVARLKNNNRQVCIDPKLKWIQEYLEKALNK

SEQ ID NO: 6 - protein, 89 aa, Homo sapiens
MNAKVVVVLVLVLTALCLSDGKPVSLSYRCPCRFFESHVARANVKHLKILNTPNCALQIVARLKNNNRQVCIDPKLKWIQEYLEKALNK

SEQ ID NO: 7 - DNA, 386 bp, Mus musculus
  CDS (3)..(380)
ccatggcaaaattttggaagaaagcactattaacaattgcagccttaacagtcggcacctccgcaggaattacaagcgtttctgccagcccaaatccaggggtcgccagatctcacggcgaccagcacctggctcctaggagatggctcctggaaggcggccaagaatgtgagtgcaaagattggttcctgcaagccccgaagagaaaagccacagctgtgctggggccaccaagaaagcagtgcccctgtgatcatgtgaagggcagagaaaagaaaaatagacaccaaaagcaccacagaaagagccaaagaccctccagagcctgccagcaatttctcaaaaggtgtcacctagccagctttgctctgcctttgtagctcgag

SEQ ID NO: 8 - protein, 125 aa, Mus musculus
MAKFWKKALLTIAALTVGTSAGITSVSASPNPGVARSHGDQHLAPRRWLLEGGQECECKDWFLQAPKRKATAVLGPPRKQCPCDHVKGREKKNRHQKHHRKSQRPSRACQQFLKRCHLASFALPL

SEQ ID NO: 9 - protein, 119 aa, Mus musculus
MKLLASPFLLLLPVMLMSMVFSSPNPGVARSHGDQHLAPRRWLLEGGQECECKDWFLQAPKRKATAVLGPPRKQCPCDHVKGREKKNRHQKHHRKSQRPSRACQQFLKRCHLASFALPL

SEQ ID NO: 10 - DNA, 386 bp, Homo sapiens
  CDS (3)..(380)
ccatggcaaaattttggaagaaagcactattaacaattgcagccttaacagtcggcacctccgcaggaattacaagcgtttctgcctcattaaatccaggagtagcacggggtcatcgagatcggggacaagcaagtcggcgttggttacaagaaggtggtcaagaatgtgaatgtaaagattggtttttacgtgctccacgtcggaagtttatgactgttagtggtcttccaaagaaacaatgtccttgtgatcattttaagggaaatgttaagaaaactcgacaccaacgtcatcaccggaaacctaataagcattcacgggcatgtcaacaatttcttaaacaatgtcaacttcgttcttttgctcttcctctttaactcgag

SEQ ID NO: 11 - protein, 125 aa, Homo sapiens
MAKFWKKALLTIAALTVGTSAGITSVSASLNPGVARGHRDRGQASRRWLQEGGQECECKDWFLRAPRRKFMTVSGLPKKQCPCDHFKGNVKKTRHQRHHRKPNKHSRACQQFLKQCQLRSFALPL

SEQ ID NO: 12 - protein, 119 aa, Homo sapiens
MKVLISSLLLLLPLMLMSMVSSSLNPGVARGHRDRGQASRRWLQEGGQECECKDWFLRAPRRKFMTVSGLPKKQCPCDHFKGNVKKTRHQRHHRKPNKHSRACQQFLKQCQLRSFALPL

SEQ ID NO: 13 - DNA, 1226 bp, Mus musculus
  CDS (3)..(1220)
ccatggcaaaattttggaagaaagcactattaacaattgcagccttaacagtcggcacctccgcaggaattacaagcgtttctgcctaccaacttatgtgttactacacttcatgggctaaagatcgtccaattgaaggttcttttaagccaggaaatattgatccttgtctttgtacacatcttatttacgcttttgctggtatgcaaaataatgaaattacttacacacacgaacaagatttacgtgattacgaagctcttaatggtcttaaggataagaatactgaacttaagacacttcttgcaattggtggatggaagtttggaccagctccttttagtgcaatggtttcaactccacaaaatcggcaaatttttattcaaagtgtaattcggtttttacggcaatacaattttgatggacttaatcttgattggcaatacccaggtagtcgaggatcaccacctaaggataagcatttatttagtgttcttgtaaaagaaatgcgaaaggcttttgaagaagaaagtgttgaaaaggatattccacgtcttcttcttactagtacaggtgcaggaattattgatgtaattaagtcaggttacaagattccagaacttagtcaatcacttgattacattcaagttatgacttacgatttacacgatcctaaggatggttacacaggagaaaattctccactttacaagagtccttacgatattggaaagagtgctgatcttaatgttgattctattattagttactggaaagatcatggagctgcatcagaaaagcttattgttggttttccagcttacggacacacttttattctttcagatccatctaagacaggtattggagcacctactatttctacaggtccacctggaaagtatactgatgaaagtggtcttttagcttactacgaagtttgtacatttttaaatgaaggagctacagaagtttgggatgcaccacaagaagtaccttatgcataccagggtaatgaatgggttggatacgataatgtacgtagttttaagcttaaggctcaatggcttaaggataataatttaggtggagcagttgtatggccacttgatatggatgatttttctggtagtttttgtcatcaacggcactttcctcttacttcaacacttaagggtgatcttaatattcattcagcatcttgtaagggaccatattaactcgag

SEQ ID NO: 14 - protein, 405 aa, Mus musculus
MAKFWKKALLTIAALTVGTSAGITSVSAYQLMCYYTSWAKDRPIEGSFKPGNIDPCLCTHLIYAFAGMQNNEITYTHEQDLRDYEALNGLKDKNTELKTLLAIGGWKFGPAPFSAMVSTPQNRQIFIQSVIRFLRQYNFDGLNLDWQYPGSRGSPPKDKHLFSVLVKEMRKAFEEESVEKDIPRLLLTSTGAGIIDVIKSGYKIPELSQSLDYIQVMTYDLHDPKDGYTGENSPLYKSPYDIGKSADLNVDSIISYWKDHGAASEKLIVGFPAYGHTFILSDPSKTGIGAPTISTGPPGKYTDESGLLAYYEVCTFLNEGATEVWDAPQEVPYAYQGNEWVGYDNVRSFKLKAQWLKDNNLGGAVVWPLDMDDFSGSFCHQRHFPLTSTLKGDLNIHSASCKGPY

SEQ ID NO: 15 - protein, 398 aa, Mus musculus
MAKLILVTGLAILLNVQLGSSYQLMCYYTSWAKDRPIEGSFKPGNIDPCLCTHLIYAFAGMQNNEITYTHEQDLRDYEALNGLKDKNTELKTLLAIGGWKFGPAPFSAMVSTPQNRQIFIQSVIRFLRQYNFDGLNLDWQYPGSRGSPPKDKHLFSVLVKEMRKAFEEESVEKDIPRLLLTSTGAGIIDVIKSGYKIPELSQSLDYIQVMTYDLHDPKDGYTGENSPLYKSPYDIGKSADLNVDSIISYWKDHGAASEKLIVGFPAYGHTFILSDPSKTGIGAPTISTGPPGKYTDESGLLAYYEVCTFLNEGATEVWDAPQEVPYAYQGNEWVGYDNVRSFKLKAQWLKDNNLGGAVVWPLDMDDFSGSFCHQRHFPLTSTLKGDLNIHSASCKGPY

SEQ ID NO: 16 - DNA, 1181 bp, Homo sapiens
  CDS (3)..(1175)
ccatggcaaaattttggaagaaagcactattaacaattgcagccttaacagtcggcacctccgcaggaattacaagcgtttctgcctacaagcttgtttgttactacacttcatggtctcaataccgagaaggtgatggaagttgttttccagatgctcttgatcggtttttatgtacacatattatttactcttttgcaaatattagtaatgatcacattgatacatgggaatggaatgatgttactctttacggtatgcttaatacacttaagaatcgtaatccaaatttaaagactttacttagtgtaggtggatggaattttggttctcaacggtttagtaagattgcttcaaatactcaatctcgtcggacatttattaaaagtgttccaccatttttacgtactcatggttttgatggacttgatttagcatggctttatccaggtcgacgtgataagcaacactttactacacttattaaagaaatgaaggctgaatttattaaggaagcacaacctggtaaaaagcaacttcttcttagtgctgcattatcagctggaaaggttactattgatagttcatacgatattgcaaagattagtcaacatcttgattttatttcaattatgacatacgattttcacggtgcttggcggggtactacaggacatcacagtccattatttcgtggacaagaagatgcttcacctgatcggttttctaatactgattatgcagttggttacatgcttcggttaggagctccagcatctaaacttgtaatgggtattcctacttttggacgatcatttacattagcttctagtgaaactggtgttggagcaccaatttcaggtccaggaattcctggtcgttttactaaggaagctggaacacttgcatactacgaaatttgtgattttcttcggggtgctactgttcatcgaacacttggacaacaagtaccttatgcaactaaaggtaatcaatgggttggatacgatgatcaagaaagtgttaagtcaaaggtacaataccttaaggatcgacaattagctggtgcaatggtatgggctcttgatcttgatgattttcaaggtagtttttgtggacaagatcttcgttttccacttactaatgctattaaggatgcattagctgcaacataactcgag

SEQ ID NO: 17 - protein, 390 aa, Homo sapiens
MAKFWKKALLTIAALTVGTSAGITSVSAYKLVCYYTSWSQYREGDGSCFPDALDRFLCTHIIYSFANISNDHIDTWEWNDVTLYGMLNTLKNRNPNLKTLLSVGGWNFGSQRFSKIASNTQSRRTFIKSVPPFLRTHGFDGLDLAWLYPGRRDKQHFTTLIKEMKAEFIKEAQPGKKQLLLSAALSAGKVTIDSSYDIAKISQHLDFISIMTYDFHGAWRGTTGHHSPLFRGQEDASPDRFSNTDYAVGYMLRLGAPASKLVMGIPTFGRSFTLASSETGVGAPISGPGIPGRFTKEAGTLAYYEICDFLRGATVHRTLGQQVPYATKGNQWVGYDDQESVKSKVQYLKDRQLAGAMVWALDLDDFQGSFCGQDLRFPLTNAIKDALAAT

SEQ ID NO: 18 - protein, 383 aa, Homo sapiens
MGVKASQTGFVVLVLLQCCSAYKLVCYYTSWSQYREGDGSCFPDALDRFLCTHIIYSFANISNDHIDTWEWNDVTLYGMLNTLKNRNPNLKTLLSVGGWNFGSQRFSKIASNTQSRRTFIKSVPPFLRTHGFDGLDLAWLYPGRRDKQHFTTLIKEMKAEFIKEAQPGKKQLLLSAALSAGKVTIDSSYDIAKISQHLDFISIMTYDFHGAWRGTTGHHSPLFRGQEDASPDRFSNTDYAVGYMLRLGAPASKLVMGIPTFGRSFTLASSETGVGAPISGPGIPGRFTKEAGTLAYYEICDFLRGATVHRTLGQQVPYATKGNQWVGYDDQESVKSKVQYLKDRQLAGAMVWALDLDDFQGSFCGQDLRFPLTNAIKDALAAT

SEQ ID NO: 19 - protein, 20 aa, Lactobacillus
MAGNSSNFIHKIIKQIFTHR

SEQ ID NO: 20 - DNA, 7673 bp, artificial
  Recombinant plasmid
  CDS (5853)..(7658)
gaattcggtaccccgggttcgaaggcgccaagcttcaaattacagcacgtgttgctttgattgatagccaaaaagcagcagttgataaagcaattactgatattgctgaaaaattgtaatttataaataaaaatcaccttttagaggtggtttttttatttataaattattcgtttgatttcgctttcgatagaacaatcaaagcgagaataaggaagataaatcccataagggcgggagcagaatgtccgagactaattcatgagatcgattttttattaaaacgtctcaaaatcgtttctgagacgttttagcgtttatttcgtttagttatcggcataatcgttaaaacaggcgttatcgtagcgtaaaagcccttgagcgtagcgtgctttgcagcgaagatgttgtctgttagattatgaaagccgatgactgaatgaaataataagcgcagcgtccttctatttcggttggaggaggctcaagggagtttgagggaatgaaattccctcatgggtttgattttaaaaattgcttgcaattttgccgagcggtagcgctggaaaaatttttgaaaaaaatttggaatttggaaaaaaatggggggaaaggaagcgaattttgcttccgtactacgaccccccattaagtgccgagtgccaatttttgtgccaaaaacgctctatcccaactggctcaagggtttgaggggtttttcaatcgccaacgaatcgccaacgttttcgccaacgttttttataaatctatatttaagtagctttattgttgtttttatgattacaaagtgatacactaattttataaaattatttgattggagttttttaaatggtgatttcagaatcgaaaaaaagagttatgatttctctgacaaaagagcaagataaaaaattaacagatatggcgaaacaaaaaggtttttcaaaatctgcggttgcggcgttagctatagaagaatatgcaagaaaggaatcagaataaaaaaaataagcgaaagctcgcgtttttagaaggatacgagttttcgctacttgtttttgataaggtaatatatcatggctattaaatactaaagctagaaattttggatttttattatatcctgactcaattcctaatgattggaaagaaaaattagagagtttgggcgtatctatggctgtcagtcctttacacgatatggacgaaaaaaaagataaagatacatggaatagtagtgatgttatacgaaatggaaagcactataaaaaaccacactatcacgttatatatattgcacgaaatcctgtaacaatagaaagcgttaggaacaagattaagcgaaaattggggaatagttcagttgctcatgttgagatacttgattatatcaaaggttcatatgaatatttgactcatgaatcaaaggacgctattgctaagaataaacatatatacgacaaaaaagatattttgaacattaatgattttgatattgaccgctatataacacttgatgaaagccaaaaaagagaattgaagaatttacttttagatatagtggatgactataatttggtaaatacaaaagatttaatggcttttattcgccttaggggagcggagtttggaattttaaatacgaatgatgtaaaagatattgtttcaacaaactctagcgcctttagattatggtttgagggcaattatcagtgtggatatagagcaagttatgcaaaggttcttgatgctgaaacgggggaaataaaatgacaaacaaagaaaaagagttatttgctgaaaatgaggaattaaaaaaagaaattaaggacttaaaagagcgtattgaaagatacagagaaatggaagttgaattaagtacaacaatagatttattgagaggagggattattgaataaataaaagcccccctgacgaaagtcgaagggggcttttattttggtttgatgttgcgattaatagcaatacgattgcaataaacaaaatgatccccttagaagcaaacttaagagtgtgttgatagtgcattatcttaaaattttgtataataggaattgaagttaaattagatgctaaaaataggaattgaagttaaattagatgctaaaaatttgtaattaagaaggagggattcgtcatgttggtattccaaatgcgtaatgtagataaaacatctactgttttgaaacagactaaaaacagtgattacgcagataaataaatacgttagattaattcctaccagtgactaatcttatgactttttaaacagataactaaaattacaaacaaatcgtttaacttcaggagagattacatgaacaaaaatataaatatctcaaactttttaacgagtgaaaaagtactcaaccaaataataaaacaattgaatttaaaagaaaccgataccgtttacgaaattggaacaggtaaagggcatttaacgacgaaactggctaaaataagtaaacaggtaacgtctattgaattagacagtcatctattcaacttatcgtcagaaaaattaaaactgaatactcgtgtcactttaattcaccaagatattctacagtttcaattccctaacaaacagaggtataaaattgttgggaatattccttacaatttaagcacacaaattattaaaaaagtggtttttgaaagccgtgcgtctgacatctatctgactgttgaagaaggattctacaagcgtaccttggatattcaccgaacactagggttgctcttgcacactcaagtctcgattcagcaattgcttaagctgccagcggaatgctttcatcctaaaccaaaagtaaacagtgtcttaataaaacttacccgccataccacagatgttccagataaatattggaagctatataagtactttgtttcaaaatgggtcaatcgagaatatcgtcaactgtttactaaaaatcagtttcgtcaagcaatgaaacacgccaaagtaaacaatttaagtaccattacttatgagcaagtattgtctatttttaatagttatctattatttaacgggaggaaataattctatgagtcgcttttttaaatttggaaagttacacgttactaaagggaatggagaccggggtcgacccttcaatagagttcttaacgttaatccgaaaaaaactaacgttaatattaaaaaataagatccgcttgtgaattatgtataatttgattagactaaagaataggagaaagtatgatgatatttaaaaaactttctcgttaagataggttgttggtgagcatgttatatacggatgtatcggtttccttaatgcaaaattttgttgctatcttattaatttttctattatatagatatattcaaagaaagataacatttaaacggatcatattagatattttaatagcgattattttttcaatattatatctgtttatttcagatgcgtcattacttgtaatggtattaatgcgattagggtggcattttcatcaacaaaaagaaaataagataaaaacgactgatacagctaatttaattctaattatcgtgatccagttattgttagttgcggttgggactattattagtcagtttaccatatcgattatcaaaagtgatttcagccaaaatatattgaacaatagtgcaacagatataactttattaggtattttctttgctgttttatttgacggcttgttctttatattattgaagaataagcggactgaattacaacatttaaatcaagaaatcattgaattttcgttagaaaaacaatattttatatttatatttattttatttatagtaatagaaattattttagcagttgggaatcttcaaggagtaacagccacgatattattaaccattatcattattttttgtgtccttatcgggatgactttttggcaagtgatgctttttttgaaggcttattcgattcgccaagaagccaatgaccaattggtccggaatcaacaacttcaagattatctagtcaatatcgaacagcagtacaccgaattacggcgatttaagcatgattatcaaaacatcttattatcgttggagagttttgccgaaaagggcgatcagcaacagtttaaggcgtattaccaagaattattagcacaacggccaattcaaagtgaaatccaaggggcagtcattgcacaactcgactacttgaaaaatgatcctattcgaggattagtcattcaaaagtttttggcagccaaacaggctggtgttactttaaaattcgaaatgaccgaaccaatcgaattagcaaccgctaatctattaacggttattcggattatcggtattttattagacaatgcgattgaacaagccgttcaagaaaccgatcaattggtgagttgtgctttcttacaatctgatggtttaatcgaaattacgattgaaaatacggccagtcaagttaagaatctccaagcattttcagagttaggctattcaacgaaaggcgctggtcgggggactggtttagctaatgtgcaggatttgattgccaaacaaaccaatttattcttagaaacacagattgaaaatagaaagttacgacagacattgatgattacggaggaaacttaatttgtatcccgtttatttattagaggatgatttacagcaacaagcgatttatcagcaaattatcgcgaatacgattatgattaacgaatttgcaatgactttaacatgcgctgccagtgatactgagacattgttggcggcaattaaggatcagcaacgaggtttattctttttggatatggaaattgaggataaccgccaagccggtttagaagtggcaactaagattcggcagatgatgccgtttgcgcaaattgtcttcattacaacccacgaggaactgacattattaacgttagaacgaaaaatagcgcctttagattacattctcaaggaccaaacaatggctgaaatcaaaaggcaattgattgatgatctattgttagctgagaagcaaaacgaggcggcagcgtatcaccgagaaaatttatttagttataaaataggtcctcgctttttctcattaccattaaaggaagttgtttatttatatactgaaaaagaaaatccgggtcatattaatttgttagccgttaccagaaaggttacttttccaggaaatttaaatgcgctggaagcccaatatccaatgctctttcggtgtgataaaagttacttagttaacctatctaatattgccaattatgacagtaaaacacggagtttaaaatttgtagatggcagtgaggcaaaagtctcgttccggaaatcacgggaactagtggccaaattaaaacaaatgatgtagcgcctgcaggcacgccaaatgatcccagtaaaaagccacccgcatggcgggtggctttttattagccctagaagggcttcccacacgcatttcagcgccttagtgccttagtttgtgaatcataggtggtatagtcccgaaatacccgtctaaggaattgtcagataggcctaatgactggcttttataatatgagataatgccgactgtactttttacagtcggttttctaatgtcactaacctgccccgttagttgaagaaggtttttatattacagctccagatctaccggtttaatttgaaaattgatattagcgtttaacagttaaattaatacgttaataatttttttgtctttaaatagggatttgaagcataatggtgttatagcgtacttagctggccagcatatatgtattctataaaatactattacaaggagattttagccatggtacgtcctgtagaaaccccaacccgtgaaatcaaaaaactcgacggcctgtgggcattcagtctggatcgcgaaaactgtggaattgatcagcgttggtgggaaagcgcgttacaagaaagccgggcaattgctgtgccaggcagttttaacgatcagttcgccgatgcagatattcgtaattatgcgggcaacgtctggtatcagcgcgaagtctttataccgaaaggttgggcaggccagcgtatcgtgctgcgtttcgatgcggtcactcattacggcaaagtgtgggtcaataatcaggaagtgatggagcatcagggcggctatacgccatttgaagccgatgtcacgccgtatgttattgccgggaaaagtgtacgtatcaccgtttgtgtgaacaacgaactgaactggcagactatcccgccgggaatggtgattaccgacgaaaacggcaagaaaaagcagtcttacttccatgatttctttaactatgccggaatccatcgcagcgtaatgctctacaccacgccgaacacctgggtggacgatatcaccgtggtgacgcatgtcgcgcaagactgtaaccacgcgtctgttgactggcaggtggtggccaatggtgatgtcagcgttgaactgcgtgatgcggatcaacaggtggttgcaactggacaaggcactagcgggactttgcaagtggtgaatccgcacctctggcaaccgggtgaaggttatctctatgaactgtgcgtcacagccaaaagccagacagagtgtgatatctacccgcttcgcgtcggcatccggtcagtggcagtgaagggcgaacagttcctgattaaccacaaaccgttctactttactggctttggtcgtcatgaagatgcggacttgcgtggcaaaggattcgataacgtgctgatggtgcacgaccacgcattaatggactggattggggccaactcctaccgtacctcgcattacccttacgctgaagagatgctcgactgggcagatgaacatggcatcgtggtgattgatgaaactgctgctgtcggctttaacctctctttaggcattggtttcgaagcgggcaacaagccgaaagaactgtacagcgaagaggcagtcaacggggaaactcagcaagcgcacttacaggcgattaaagagctgatagcgcgtgacaaaaaccacccaagcgtggtgatgtggagtattgccaacgaaccggatacccgtccgcaaggtgcacgggaatatttcgcgccactggcggaagcaacgcgtaaactcgacccgacgcgtccgatcacctgcgtcaatgtaatgttctgcgacgctcacaccgataccatcagcgatctctttgatgtgctgtgcctgaaccgttattacggatggtatgtccaaagcggcgatttggaaacggcagagaaggtactggaaaaagaacttctggcctggcaggagaaactgcatcagccgattatcatcaccgaatacggcgtggatacgttagccgggctgcactcaatgtacaccgacatgtggagtgaagagtatcagtgtgcatggctggatatgtatcaccgcgtctttgatcgcgtcagcgccgtcgtcggtgaacaggtatggaatttcgccgattttgcgacctcgcaaggcatattgcgcgttggcggtaacaagaaagggatcttcactcgcgaccgcaaaccgaagtcggcggcttttctgctgcaaaaacgctggactggcatgaacttcggtgaaaaaccgcagggaggcaaacaatgatctagactcgag

SEQ ID NO: 21 - protein, 602 aa, artificial
  Synthetic Construct
MVRPVETPTREIKKLDGLWAFSLDRENCGIDQRWWESALQESRAIAVPGSFNDQFADADIRNYAGNVWYQREVFIPKGWAGQRIVLRFDAVTHYGKVWVNNQEVMEHQGGYTPFEADVTPYVIAGKSVRITVCVNNELNWQTIPPGMVITDENGKKKQSYFHDFFNYAGIHRSVMLYTTPNTWVDDITVVTHVAQDCNHASVDWQVVANGDVSVELRDADQQVVATGQGTSGTLQVVNPHLWQPGEGYLYELCVTAKSQTECDIYPLRVGIRSVAVKGEQFLINHKPFYFTGFGRHEDADLRGKGFDNVLMVHDHALMDWIGANSYRTSHYPYAEEMLDWADEHGIVVIDETAAVGFNLSLGIGFEAGNKPKELYSEEAVNGETQQAHLQAIKELIARDKNHPSVVMWSIANEPDTRPQGAREYFAPLAEATRKLDPTRPITCVNVMFCDAHTDTISDLFDVLCLNRYYGWYVQSGDLETAEKVLEKELLAWQEKLHQPIIITEYGVDTLAGLHSMYTDMWSEEYQCAWLDMYHRVFDRVSAVVGEQVWNFADFATSQGILRVGGNKKGIFTRDRKPKSAAFLLQKRWTGMNFGEKPQGGKQ

SEQ ID NO: 22 - DNA, 22 bp, artificial
  PCR primer
gcagccttaacagtcggcacct

SEQ ID NO: 23 - DNA, 23 bp, artificial
  PCR primer
acgtgcaacaatctgcaaagcac

SEQ ID NO: 24 - DNA, 2999 bp, artificial
  pVAX vector
gactcttcgcgatgtacgggccagatatacgcgttgacattgattattgactagttattaatagtaatcaattacggggtcattagttcatagcccatatatggagttccgcgttacataacttacggtaaatggcccgcctggctgaccgcccaacgacccccgcccattgacgtcaataatgacgtatgttcccatagtaacgccaatagggactttccattgacgtcaatgggtggactatttacggtaaactgcccacttggcagtacatcaagtgtatcatatgccaagtacgccccctattgacgtcaatgacggtaaatggcccgcctggcattatgcccagtacatgaccttatgggactttcctacttggcagtacatctacgtattagtcatcgctattaccatggtgatgcggttttggcagtacatcaatgggcgtggatagcggtttgactcacggggatttccaagtctccaccccattgacgtcaatgggagtttgttttggcaccaaaatcaacgggactttccaaaatgtcgtaacaactccgccccattgacgcaaatgggcggtaggcgtgtacggtgggaggtctatataagcagagctctctggctaactagagaacccactgcttactggcttatcgaaattaatacgactcactatagggagacccaagctggctagcgtttaaacttaagcttggtaccgagctcggatccactagtccagtgtggtggaattctgcagatatccagcacagtggcggccgctcgagtctagagggcccgtttaaacccgctgatcagcctcgactgtgccttctagttgccagccatctgttgtttgcccctcccccgtgccttccttgaccctggaaggtgccactcccactgtcctttcctaataaaatgaggaaattgcatcgcattgtctgagtaggtgtcattctattctggggggtggggtggggcaggacagcaagggggaggattgggaagacaatagcaggcatgctggggatgcggtgggctctatggcttctactgggcggttttatggacagcaagcgaaccggaattgccagctggggcgccctctggtaaggttgggaagccctgcaaagtaaactggatggctttctcgccgccaaggatctgatggcgcaggggatcaagctctgatcaagagacaggatgaggatcgtttcgcatgattgaacaagatggattgcacgcaggttctccggccgcttgggtggagaggctattcggctatgactgggcacaacagacaatcggctgctctgatgccgccgtgttccggctgtcagcgcaggggcgcccggttctttttgtcaagaccgacctgtccggtgccctgaatgaactgcaagacgaggcagcgcggctatcgtggctggccacgacgggcgttccttgcgcagctgtgctcgacgttgtcactgaagcgggaagggactggctgctattgggcgaagtgccggggcaggatctcctgtcatctcaccttgctcctgccgagaaagtatccatcatggctgatgcaatgcggcggctgcatacgcttgatccggctacctgcccattcgaccaccaagcgaaacatcgcatcgagcgagcacgtactcggatggaagccggtcttgtcgatcaggatgatctggacgaagagcatcaggggctcgcgccagccgaactgttcgccaggctcaaggcgagcatgcccgacggcgaggatctcgtcgtgacccatggcgatgcctgcttgccgaatatcatggtggaaaatggccgcttttctggattcatcgactgtggccggctgggtgtggcggaccgctatcaggacatagcgttggctacccgtgatattgctgaagagcttggcggcgaatgggctgaccgcttcctcgtgctttacggtatcgccgctcccgattcgcagcgcatcgccttctatcgccttcttgacgagttcttctgaattattaacgcttacaatttcctgatgcggtattttctccttacgcatctgtgcggtatttcacaccgcatacaggtggcacttttcggggaaatgtgcgcggaacccctatttgtttatttttctaaatacattcaaatatgtatccgctcatgagacaataaccctgataaatgcttcaataatagcacgtgctaaaacttcatttttaatttaaaaggatctaggtgaagatcctttttgataatctcatgaccaaaatcccttaacgtgagttttcgttccactgagcgtcagaccccgtagaaaagatcaaaggatcttcttgagatcctttttttctgcgcgtaatctgctgcttgcaaacaaaaaaaccaccgctaccagcggtggtttgtttgccggatcaagagctaccaactctttttccgaaggtaactggcttcagcagagcgcagataccaaatactgtccttctagtgtagccgtagttaggccaccacttcaagaactctgtagcaccgcctacatacctcgctctgctaatcctgttaccagtggctgctgccagtggcgataagtcgtgtcttaccgggttggactcaagacgatagttaccggataaggcgcagcggtcgggctgaacggggggttcgtgcacacagcccagcttggagcgaacgacctacaccgaactgagatacctacagcgtgagctatgagaaagcgccacgcttcccgaagggagaaaggcggacaggtatccggtaagcggcagggtcggaacaggagagcgcacgagggagcttccagggggaaacgcctggtatctttatagtcctgtcgggtttcgccacctctgacttgagcgtcgatttttgtgatgctcgtcaggggggcggagcctatggaaaaacgccagcaacgcggcctttttacggttcctgggcttttgctggccttttgctcacatgttctt

SEQ ID NO: 25 - DNA, 347 bp, artificial
  insert
gctagcatggacgccaaggtcgtcgccgtgctggccctggtgctggccgcgctctgcatcagtgacggtaaaccagtcagcctgagctaccgatgcccctgccggttcttcgagagccacatcgccagagccaacgtcaagcatctgaaaatcctcaacactccaaactgtgcccttcagattgttgcacggctgaagaacaacaacagacaagtgtgcattgacccgaaattaaagtggatccaagagtacctggagaaagccttaaacaagggatcaggtgccacgaacttctctctgttaaagcaagcaggagacgtggaagaaaaccccggtcccaaaagctt

SEQ ID NO: 26 - DNA, 5395 bp, artificial
  vector
gactcttcgcgatgtacgggccagatatacgcgttgacattgattattgactagttattaatagtaatcaattacggggtcattagttcatagcccatatatggagttccgcgttacataacttacggtaaatggcccgcctggctgaccgcccaacgacccccgcccattgacgtcaataatgacgtatgttcccatagtaacgccaatagggactttccattgacgtcaatgggtggactatttacggtaaactgcccacttggcagtacatcaagtgtatcatatgccaagtacgccccctattgacgtcaatgacggtaaatggcccgcctggcattatgcccagtacatgaccttatgggactttcctacttggcagtacatctacgtattagtcatcgctattaccatggtgatgcggttttggcagtacatcaatgggcgtggatagcggtttgactcacggggatttccaagtctccaccccattgacgtcaatgggagtttgttttggcaccaaaatcaacgggactttccaaaatgtcgtaacaactccgccccattgacgcaaatgggcggtaggcgtgtacggtgggaggtctatataagcagagctctctggctaactagagaacccactgcttactggcttatcgaaattaatacgactcactatagggagacccaagctggctagcgtttaaacttaagcttcgccaccatggagagcgacgagagcggcctgcccgccatggagatcgagtgccgcatcaccggcaccctgaacggcgtggagttcgagctggtgggcggcggagagggcacccccaagcagggccgcatgaccaacaagatgaagagcaccaaaggcgccctgaccttcagcccctacctgctgagccacgtgatgggctacggcttctaccacttcggcacctaccccagcggctacgagaaccccttcctgcacgccatcaacaacggcggctacaccaacacccgcatcgagaagtacgaggacggcggcgtgctgcacgtgagcttcagctaccgctgcgaggccggccgcgtgatcggcgacttcaaggtggtgggcaccggcttccccgaggacagcgtgatcttcaccgacaagatcatccgcagcaacgccaccgtggagcacctgcaccccatgggcgataacgtgctggtgggcagcttcgcccgcaccttcagcctgcgcgacggcggctaccacagcttcgtggtggacaaccacatgcacttcaagagcgccatccaccccagcatcctgcagaacgggggccccatgttcgccttccgccgcgtggaggagctgcacagcaacaccgagctgggcatcgtggagtaccagcacgccttcaagacccccatcgccttcgccagatcccgcgctcagtcgtccaattctgccgtggacggcaccgccggacccggctccaccggatctcgcgagggcagaggaagtcttctaacatgcggtgacgtggaggagaatcccggccctatggaagatgccaaaaacattaagaagggcccagcgccattctacccactcgaagacgggaccgccggcgagcagctgcacaaagccatgaagcgctacgccctggtgcccggcaccatcgcctttaccgacgcacatatcgaggtggacattacctacgccgagtacttcgagatgagcgttcggctggcagaagctatgaagcgctatgggctgaatacaaaccatcggatcgtggtgtgcagcgagaatagcttgcagttcttcatgcccgtgttgggtgccctgttcatcggtgtggctgtggccccagctaacgacatctacaacgagcgcgagctgctgaacagcatgggcatcagccagcccaccgtcgtattcgtgagcaagaaagggctgcaaaagatcctcaacgtgcaaaagaagctaccgatcatacaaaagatcatcatcatggatagcaagaccgactaccagggcttccaaagcatgtacaccttcgtgacttcccatttgccacccggcttcaacgagtacgacttcgtgcccgagagcttcgaccgggacaaaaccatcgccctgatcatgaacagtagtggcagtaccggattgcccaagggcgtagccctaccgcaccgcaccgcttgtgtccgattcagtcatgcccgcgaccccatcttcggcaaccagatcatccccgacaccgctatcctcagcgtggtgccatttcaccacggcttcggcatgttcaccacgctgggctacttgatctgcggctttcgggtcgtgctcatgtaccgcttcgaggaggagctattcttgcgcagcttgcaagactataagattcaatctgccctgctggtgcccacactatttagcttcttcgctaagagcactctcatcgacaagtacgacctaagcaacttgcacgagatcgccagcggcggggcgccgctcagcaaggaggtaggtgaggccgtggccaaacgcttccacctaccaggcatccgccagggctacggcctgacagaaacaaccagcgccattctgatcacccccgaaggggacgacaagcctggcgcagtaggcaaggtggtgcccttcttcgaggctaaggtggtggacttggacaccggtaagacactgggtgtgaaccagcgcggcgagctgtgcgtccgtggccccatgatcatgagcggctacgttaacaaccccgaggctacaaacgctctcatcgacaaggacggctggctgcacagcggcgacatcgcctactgggacgaggacgagcacttcttcatcgtggaccggctgaagagcctgatcaaatacaagggctaccaggtagccccagccgaactggagagcatcctgctgcaacaccccaacatcttcgacgccggggtcgccggcctgcccgacgacgatgccggcgagctgcccgccgcagtcgtcgtgctggaacacggtaaaaccatgaccgagaaggagatcgtggactatgtggccagccaggttacaaccgccaagaagctgcgcggtggtgttgtgttcgtggacgaggtgcctaaaggactgaccggcaagttggacgcccgcaagatccgcgagattctcattaaggccaagaagggcggcaagatcgccgtgtaatctagagggcccgtttaaacccgctgatcagcctcgactgtgccttctagttgccagccatctgttgtttgcccctcccccgtgccttccttgaccctggaaggtgccactcccactgtcctttcctaataaaatgaggaaattgcatcgcattgtctgagtaggtgtcattctattctggggggtggggtggggcaggacagcaagggggaggattgggaagacaatagcaggcatgctggggatgcggtgggctctatggcttctactgggcggttttatggacagcaagcgaaccggaattgccagctggggcgccctctggtaaggttgggaagccctgcaaagtaaactggatggctttctcgccgccaaggatctgatggcgcaggggatcaagctctgatcaagagacaggatgaggatcgtttcgcatgattgaacaagatggattgcacgcaggttctccggccgcttgggtggagaggctattcggctatgactgggcacaacagacaatcggctgctctgatgccgccgtgttccggctgtcagcgcaggggcgcccggttctttttgtcaagaccgacctgtccggtgccctgaatgaactgcaagacgaggcagcgcggctatcgtggctggccacgacgggcgttccttgcgcagctgtgctcgacgttgtcactgaagcgggaagggactggctgctattgggcgaagtgccggggcaggatctcctgtcatctcaccttgctcctgccgagaaagtatccatcatggctgatgcaatgcggcggctgcatacgcttgatccggctacctgcccattcgaccaccaagcgaaacatcgcatcgagcgagcacgtactcggatggaagccggtcttgtcgatcaggatgatctggacgaagagcatcaggggctcgcgccagccgaactgttcgccaggctcaaggcgagcatgcccgacggcgaggatctcgtcgtgacccatggcgatgcctgcttgccgaatatcatggtggaaaatggccgcttttctggattcatcgactgtggccggctgggtgtggcggaccgctatcaggacatagcgttggctacccgtgatattgctgaagagcttggcggcgaatgggctgaccgcttcctcgtgctttacggtatcgccgctcccgattcgcagcgcatcgccttctatcgccttcttgacgagttcttctgaattattaacgcttacaatttcctgatgcggtattttctccttacgcatctgtgcggtatttcacaccgcatacaggtggcacttttcggggaaatgtgcgcggaacccctatttgtttatttttctaaatacattcaaatatgtatccgctcatgagacaataaccctgataaatgcttcaataatagcacgtgctaaaacttcatttttaatttaaaaggatctaggtgaagatcctttttgataatctcatgaccaaaatcccttaacgtgagttttcgttccactgagcgtcagaccccgtagaaaagatcaaaggatcttcttgagatcctttttttctgcgcgtaatctgctgcttgcaaacaaaaaaaccaccgctaccagcggtggtttgtttgccggatcaagagctaccaactctttttccgaaggtaactggcttcagcagagcgcagataccaaatactgtccttctagtgtagccgtagttaggccaccacttcaagaactctgtagcaccgcctacatacctcgctctgctaatcctgttaccagtggctgctgccagtggcgataagtcgtgtcttaccgggttggactcaagacgatagttaccggataaggcgcagcggtcgggctgaacggggggttcgtgcacacagcccagcttggagcgaacgacctacaccgaactgagatacctacagcgtgagctatgagaaagcgccacgcttcccgaagggagaaaggcggacaggtatccggtaagcggcagggtcggaacaggagagcgcacgagggagcttccagggggaaacgcctggtatctttatagtcctgtcgggtttcgccacctctgacttgagcgtcgatttttgtgatgctcgtcaggggggcggagcctatggaaaaacgccagcaacgcggcctttttacggttcctgggcttttgctggccttttgctcacatgttctt